European Patent Specification EP 4 003 400 B1, published April 3, 2024. Title: DOSING FOR PREVENTION OR TREATMENT OF GRAFT VERSUS HOST DISEASE (GVHD) WITH IL-22 Fc FUSION PROTEINS. Applicant: Genentech, Inc. The sequence listing filed with the application follows.

SEQUENCE LISTING (80 sequences)

SEQ ID NO: 1 - DNA, 495 bp, Homo sapiens
  Human IL-22
atgggatggtcatgtatcatcctttttctagtagcaactgcaactggagtacattcagcgcccatcagctcccactgcaggcttgacaagtccaacttccagcagccctatatcaccaaccgcaccttcatgctggctaaggaggctagcttggctgataacaacacagacgttcgtctcattggggagaaactgttccacggagtcagtatgagtgagcgctgctatctgatgaagcaggtgctgaacttcacccttgaagaagtgctgttccctcaatctgataggttccagccttatatgcaggaggtggtgcccttcctggccaggctcagcaacaggctaagcacatgtcatattgaaggtgatgacctgcatatccagaggaatgtgcaaaagctgaaggacacagtgaaaaagcttggagagagtggagagatcaaagcaattggagaactggatttgctgtttatgtctctgagaaatgcctgcatt

SEQ ID NO: 2 - protein, 165 aa, Homo sapiens
  Human IL-22
MGWSCIILFLVATATGVHSAPISSHCRLDKSNFQQPYITNRTFMLAKEASLADNNTDVRLIGEKLFHGVSMSERCYLMKQVLNFTLEEVLFPQSDRFQPYMQEVVPFLARLSNRLSTCHIEGDDLHIQRNVQKLKDTVKKLGESGEIKAIGELDLLFMSLRNACI

SEQ ID NO: 3 - DNA, 438 bp, Homo sapiens
  IL-22 DNA (mature)
gcgcccatcagctcccactgcaggcttgacaagtccaacttccagcagccctatatcaccaaccgcaccttcatgctggctaaggaggctagcttggctgataacaacacagacgttcgtctcattggggagaaactgttccacggagtcagtatgagtgagcgctgctatctgatgaagcaggtgctgaacttcacccttgaagaagtgctgttccctcaatctgataggttccagccttatatgcaggaggtggtgcccttcctggccaggctcagcaacaggctaagcacatgtcatattgaaggtgatgacctgcatatccagaggaatgtgcaaaagctgaaggacacagtgaaaaagcttggagagagtggagagatcaaagcaattggagaactggatttgctgtttatgtctctgagaaatgcctgcatt

SEQ ID NO: 4 - protein, 146 aa, Homo sapiens
  IL-22 (mature)
APISSHCRLDKSNFQQPYITNRTFMLAKEASLADNNTDVRLIGEKLFHGVSMSERCYLMKQVLNFTLEEVLFPQSDRFQPYMQEVVPFLARLSNRLSTCHIEGDDLHIQRNVQKLKDTVKKLGESGEIKAIGELDLLFMSLRNACI

SEQ ID NO: 5 - DNA, 57 bp, Homo sapiens
  IL-22 leader sequence
atgggatggtcatgtatcatcctttttctagtagcaactgcaactggagtacattca

SEQ ID NO: 6 - protein, 19 aa, Homo sapiens
  IL-22 leader sequence
MGWSCIILFLVATATGVHS

SEQ ID NO: 7 - DNA, 1128 bp, Artificial Sequence
  Description of Artificial Sequence: Synthetic polynucleotide
  IL-22 Fc fusion IgG4 (minus C-terminal Lys) N297G
gcgcccatcagctcccactgcaggcttgacaagtccaacttccagcagccctatatcaccaaccgcaccttcatgctggctaaggaggctagcttggctgataacaacacagacgttcgtctcattggggagaaactgttccacggagtcagtatgagtgagcgctgctatctgatgaagcaggtgctgaacttcacccttgaagaagtgctgttccctcaatctgataggttccagccttatatgcaggaggtggtgcccttcctggccaggctcagcaacaggctaagcacatgtcatattgaaggtgatgacctgcatatccagaggaatgtgcaaaagctgaaggacacagtgaaaaagcttggagagagtggagagatcaaagcaattggagaactggatttgctgtttatgtctctgagaaatgcctgcattcgcgttgagtccaaatatggtcccccatgcccaccatgcccagcacctgagttcctggggggaccatcagtcttcctgttccccccaaaacccaaggacactctcatgatctcccggacccctgaggtcacgtgcgtggtggtggacgtgagccaggaagaccccgaggtccagttcaactggtacgtggatggcgtggaggtgcataatgccaagacaaagccgcgggaggagcagttcggaagcacgtaccgtgtggtcagcgtcctcaccgtcctgcaccaggactggctgaacggcaaggagtacaagtgcaaggtctccaacaaaggcctcccgtcctccatcgagaaaaccatctccaaagccaaagggcagccccgagagccacaggtgtacaccctgcccccatcccaggaggagatgaccaagaaccaggtcagcctgacctgcctggtcaaaggcttctaccccagcgacatcgccgtggagtgggagagcaatgggcagccggagaacaactacaagaccacgcctcccgtgctggactccgacggctccttcttcctctacagcaggctaaccgtggacaagagcaggtggcaggaggggaatgtcttctcatgctccgtgatgcatgaggctctgcacaaccactacacacagaagagcctctccctgtctctgggt

SEQ ID NO: 8 - protein, 376 aa, Artificial Sequence
  Description of Artificial Sequence: Synthetic polypeptide
  IL-22 Fc fusion IgG4 (minus C-terminal Lys) N297G
APISSHCRLDKSNFQQPYITNRTFMLAKEASLADNNTDVRLIGEKLFHGVSMSERCYLMKQVLNFTLEEVLFPQSDRFQPYMQEVVPFLARLSNRLSTCHIEGDDLHIQRNVQKLKDTVKKLGESGEIKAIGELDLLFMSLRNACIRVESKYGPPCPPCPAPEFLGGPSVFLFPPKPKDTLMISRTPEVTCVVVDVSQEDPEVQFNWYVDGVEVHNAKTKPREEQFGSTYRVVSVLTVLHQDWLNGKEYKCKVSNKGLPSSIEKTISKAKGQPREPQVYTLPPSQEEMTKNQVSLTCLVKGFYPSDIAVEWESNGQPENNYKTTPPVLDSDGSFFLYSRLTVDKSRWQEGNVFSCSVMHEALHNHYTQKSLSLSLG

SEQ ID NO: 9 - DNA, 1128 bp, Artificial Sequence
  Description of Artificial Sequence: Synthetic polynucleotide
  IL-22 Fc fusion IgG4 (minus C-terminal Lys) N297A
gcgcccatcagctcccactgcaggcttgacaagtccaacttccagcagccctatatcaccaaccgcaccttcatgctggctaaggaggctagcttggctgataacaacacagacgttcgtctcattggggagaaactgttccacggagtcagtatgagtgagcgctgctatctgatgaagcaggtgctgaacttcacccttgaagaagtgctgttccctcaatctgataggttccagccttatatgcaggaggtggtgcccttcctggccaggctcagcaacaggctaagcacatgtcatattgaaggtgatgacctgcatatccagaggaatgtgcaaaagctgaaggacacagtgaaaaagcttggagagagtggagagatcaaagcaattggagaactggatttgctgtttatgtctctgagaaatgcctgcattcgcgttgagtccaaatatggtcccccatgcccaccatgcccagcacctgagttcctggggggaccatcagtcttcctgttccccccaaaacccaaggacactctcatgatctcccggacccctgaggtcacgtgcgtggtggtggacgtgagccaggaagaccccgaggtccagttcaactggtacgtggatggcgtggaggtgcataatgccaagacaaagccgcgggaggagcagttcgctagcacgtaccgtgtggtcagcgtcctcaccgtcctgcaccaggactggctgaacggcaaggagtacaagtgcaaggtctccaacaaaggcctcccgtcctccatcgagaaaaccatctccaaagccaaagggcagccccgagagccacaggtgtacaccctgcccccatcccaggaggagatgaccaagaaccaggtcagcctgacctgcctggtcaaaggcttctaccccagcgacatcgccgtggagtgggagagcaatgggcagccggagaacaactacaagaccacgcctcccgtgctggactccgacggctccttcttcctctacagcaggctaaccgtggacaagagcaggtggcaggaggggaatgtcttctcatgctccgtgatgcatgaggctctgcacaaccactacacacagaagagcctctccctgtctctgggt

SEQ ID NO: 10 - protein, 376 aa, Artificial Sequence
  Description of Artificial Sequence: Synthetic polypeptide
  IL-22 Fc fusion IgG4 (minus C-terminal Lys) N297A
APISSHCRLDKSNFQQPYITNRTFMLAKEASLADNNTDVRLIGEKLFHGVSMSERCYLMKQVLNFTLEEVLFPQSDRFQPYMQEVVPFLARLSNRLSTCHIEGDDLHIQRNVQKLKDTVKKLGESGEIKAIGELDLLFMSLRNACIRVESKYGPPCPPCPAPEFLGGPSVFLFPPKPKDTLMISRTPEVTCVVVDVSQEDPEVQFNWYVDGVEVHNAKTKPREEQFASTYRVVSVLTVLHQDWLNGKEYKCKVSNKGLPSSIEKTISKAKGQPREPQVYTLPPSQEEMTKNQVSLTCLVKGFYPSDIAVEWESNGQPENNYKTTPPVLDSDGSFFLYSRLTVDKSRWQEGNVFSCSVMHEALHNHYTQKSLSLSLG

SEQ ID NO: 11 - DNA, 1131 bp, Artificial Sequence
  Description of Artificial Sequence: Synthetic polynucleotide
  IL-22 Fc fusion IgG1 (minus C-terminal Lys) N297G
gcgcccatcagctcccactgcaggcttgacaagtccaacttccagcagccctatatcaccaaccgcaccttcatgctggctaaggaggctagcttggctgataacaacacagacgttcgtctcattggggagaaactgttccacggagtcagtatgagtgagcgctgctatctgatgaagcaggtgctgaacttcacccttgaagaagtgctgttccctcaatctgataggttccagccttatatgcaggaggtggtgcccttcctggccaggctcagcaacaggctaagcacatgtcatattgaaggtgatgacctgcatatccagaggaatgtgcaaaagctgaaggacacagtgaaaaagcttggagagagtggagagatcaaagcaattggagaactggatttgctgtttatgtctctgagaaatgcctgcattgagcccaaatctagtgacaaaactcacacatgcccaccgtgcccagcacctgaactcctggggggaccgtcagtcttcctcttccccccaaaacccaaggacaccctcatgatctcccggacccctgaggtcacatgcgtggtggtggacgtgagccacgaagaccctgaggtcaagttcaactggtacgtggacggcgtggaggtgcataatgccaagacaaagccgcgggaggagcagtacggaagcacgtaccgtgtggtcagcgtcctcaccgtcctgcaccaggactggctgaatggcaaggagtacaagtgcaaggtctccaacaaagccctcccagcccccatcgagaaaaccatctccaaagccaaagggcagccccgagaaccacaggtgtacaccctgcccccatcccgggaagagatgaccaagaaccaggtcagcctgacctgcctggtcaaaggcttctatcccagcgacatcgccgtggagtgggagagcaatgggcagccggagaacaactacaagaccacgcctcccgtgctggactccgacggctccttcttcctctacagcaagctcaccgtggacaagagcaggtggcagcaggggaacgtcttctcatgctccgtgatgcatgaggctctgcacaaccactacacgcagaagagcctctccctgtctccgggt

SEQ ID NO: 12 - protein, 377 aa, Artificial Sequence
  Description of Artificial Sequence: Synthetic polypeptide
  IL-22 Fc fusion IgG1 (minus C-terminal Lys) N297G
APISSHCRLDKSNFQQPYITNRTFMLAKEASLADNNTDVRLIGEKLFHGVSMSERCYLMKQVLNFTLEEVLFPQSDRFQPYMQEVVPFLARLSNRLSTCHIEGDDLHIQRNVQKLKDTVKKLGESGEIKAIGELDLLFMSLRNACIEPKSSDKTHTCPPCPAPELLGGPSVFLFPPKPKDTLMISRTPEVTCVVVDVSHEDPEVKFNWYVDGVEVHNAKTKPREEQYGSTYRVVSVLTVLHQDWLNGKEYKCKVSNKALPAPIEKTISKAKGQPREPQVYTLPPSREEMTKNQVSLTCLVKGFYPSDIAVEWESNGQPENNYKTTPPVLDSDGSFFLYSKLTVDKSRWQQGNVFSCSVMHEALHNHYTQKSLSLSPG

SEQ ID NO: 13 - DNA, 1131 bp, Artificial Sequence
  Description of Artificial Sequence: Synthetic polynucleotide
  IL-22 Fc fusion IgG1 (minus C-terminal Lys) N297A
gcgcccatcagctcccactgcaggcttgacaagtccaacttccagcagccctatatcaccaaccgcaccttcatgctggctaaggaggctagcttggctgataacaacacagacgttcgtctcattggggagaaactgttccacggagtcagtatgagtgagcgctgctatctgatgaagcaggtgctgaacttcacccttgaagaagtgctgttccctcaatctgataggttccagccttatatgcaggaggtggtgcccttcctggccaggctcagcaacaggctaagcacatgtcatattgaaggtgatgacctgcatatccagaggaatgtgcaaaagctgaaggacacagtgaaaaagcttggagagagtggagagatcaaagcaattggagaactggatttgctgtttatgtctctgagaaatgcctgcattgagcccaaatctagtgacaaaactcacacatgcccaccgtgcccagcacctgaactcctggggggaccgtcagtcttcctcttccccccaaaacccaaggacaccctcatgatctcccggacccctgaggtcacatgcgtggtggtggacgtgagccacgaagaccctgaggtcaagttcaactggtacgtggacggcgtggaggtgcataatgccaagacaaagccgcgggaggagcagtacgctagcacgtaccgtgtggtcagcgtcctcaccgtcctgcaccaggactggctgaatggcaaggagtacaagtgcaaggtctccaacaaagccctcccagcccccatcgagaaaaccatctccaaagccaaagggcagccccgagaaccacaggtgtacaccctgcccccatcccgggaagagatgaccaagaaccaggtcagcctgacctgcctggtcaaaggcttctatcccagcgacatcgccgtggagtgggagagcaatgggcagccggagaacaactacaagaccacgcctcccgtgctggactccgacggctccttcttcctctacagcaagctcaccgtggacaagagcaggtggcagcaggggaacgtcttctcatgctccgtgatgcatgaggctctgcacaaccactacacgcagaagagcctctccctgtctccgggt

SEQ ID NO: 14 - protein, 377 aa, Artificial Sequence
  Description of Artificial Sequence: Synthetic polypeptide
  IL-22 Fc fusion IgG1 (minus C-terminal Lys) N297A
APISSHCRLDKSNFQQPYITNRTFMLAKEASLADNNTDVRLIGEKLFHGVSMSERCYLMKQVLNFTLEEVLFPQSDRFQPYMQEVVPFLARLSNRLSTCHIEGDDLHIQRNVQKLKDTVKKLGESGEIKAIGELDLLFMSLRNACIEPKSSDKTHTCPPCPAPELLGGPSVFLFPPKPKDTLMISRTPEVTCVVVDVSHEDPEVKFNWYVDGVEVHNAKTKPREEQYASTYRVVSVLTVLHQDWLNGKEYKCKVSNKALPAPIEKTISKAKGQPREPQVYTLPPSREEMTKNQVSLTCLVKGFYPSDIAVEWESNGQPENNYKTTPPVLDSDGSFFLYSKLTVDKSRWQQGNVFSCSVMHEALHNHYTQKSLSLSPG

SEQ ID NO: 15 - DNA, 1131 bp, Artificial Sequence
  Description of Artificial Sequence: Synthetic polynucleotide
  IL-22 Fc fusion IgG4 (full) N297G
gcgcccatcagctcccactgcaggcttgacaagtccaacttccagcagccctatatcaccaaccgcaccttcatgctggctaaggaggctagcttggctgataacaacacagacgttcgtctcattggggagaaactgttccacggagtcagtatgagtgagcgctgctatctgatgaagcaggtgctgaacttcacccttgaagaagtgctgttccctcaatctgataggttccagccttatatgcaggaggtggtgcccttcctggccaggctcagcaacaggctaagcacatgtcatattgaaggtgatgacctgcatatccagaggaatgtgcaaaagctgaaggacacagtgaaaaagcttggagagagtggagagatcaaagcaattggagaactggatttgctgtttatgtctctgagaaatgcctgcattcgcgttgagtccaaatatggtcccccatgcccaccatgcccagcacctgagttcctggggggaccatcagtcttcctgttccccccaaaacccaaggacactctcatgatctcccggacccctgaggtcacgtgcgtggtggtggacgtgagccaggaagaccccgaggtccagttcaactggtacgtggatggcgtggaggtgcataatgccaagacaaagccgcgggaggagcagttcggaagcacgtaccgtgtggtcagcgtcctcaccgtcctgcaccaggactggctgaacggcaaggagtacaagtgcaaggtctccaacaaaggcctcccgtcctccatcgagaaaaccatctccaaagccaaagggcagccccgagagccacaggtgtacaccctgcccccatcccaggaggagatgaccaagaaccaggtcagcctgacctgcctggtcaaaggcttctaccccagcgacatcgccgtggagtgggagagcaatgggcagccggagaacaactacaagaccacgcctcccgtgctggactccgacggctccttcttcctctacagcaggctaaccgtggacaagagcaggtggcaggaggggaatgtcttctcatgctccgtgatgcatgaggctctgcacaaccactacacacagaagagcctctccctgtctctgggtaaa

SEQ ID NO: 16 - protein, 377 aa, Artificial Sequence
  Description of Artificial Sequence: Synthetic polypeptide
  IL-22 Fc fusion IgG4 (full) N297G
APISSHCRLDKSNFQQPYITNRTFMLAKEASLADNNTDVRLIGEKLFHGVSMSERCYLMKQVLNFTLEEVLFPQSDRFQPYMQEVVPFLARLSNRLSTCHIEGDDLHIQRNVQKLKDTVKKLGESGEIKAIGELDLLFMSLRNACIRVESKYGPPCPPCPAPEFLGGPSVFLFPPKPKDTLMISRTPEVTCVVVDVSQEDPEVQFNWYVDGVEVHNAKTKPREEQFGSTYRVVSVLTVLHQDWLNGKEYKCKVSNKGLPSSIEKTISKAKGQPREPQVYTLPPSQEEMTKNQVSLTCLVKGFYPSDIAVEWESNGQPENNYKTTPPVLDSDGSFFLYSRLTVDKSRWQEGNVFSCSVMHEALHNHYTQKSLSLSLGK

SEQ ID NO: 17 - DNA, 1131 bp, Artificial Sequence
  Description of Artificial Sequence: Synthetic polynucleotide
  IL-22 Fc fusion IgG4 (full) N297A
gcgcccatcagctcccactgcaggcttgacaagtccaacttccagcagccctatatcaccaaccgcaccttcatgctggctaaggaggctagcttggctgataacaacacagacgttcgtctcattggggagaaactgttccacggagtcagtatgagtgagcgctgctatctgatgaagcaggtgctgaacttcacccttgaagaagtgctgttccctcaatctgataggttccagccttatatgcaggaggtggtgcccttcctggccaggctcagcaacaggctaagcacatgtcatattgaaggtgatgacctgcatatccagaggaatgtgcaaaagctgaaggacacagtgaaaaagcttggagagagtggagagatcaaagcaattggagaactggatttgctgtttatgtctctgagaaatgcctgcattcgcgttgagtccaaatatggtcccccatgcccaccatgcccagcacctgagttcctggggggaccatcagtcttcctgttccccccaaaacccaaggacactctcatgatctcccggacccctgaggtcacgtgcgtggtggtggacgtgagccaggaagaccccgaggtccagttcaactggtacgtggatggcgtggaggtgcataatgccaagacaaagccgcgggaggagcagttcgctagcacgtaccgtgtggtcagcgtcctcaccgtcctgcaccaggactggctgaacggcaaggagtacaagtgcaaggtctccaacaaaggcctcccgtcctccatcgagaaaaccatctccaaagccaaagggcagccccgagagccacaggtgtacaccctgcccccatcccaggaggagatgaccaagaaccaggtcagcctgacctgcctggtcaaaggcttctaccccagcgacatcgccgtggagtgggagagcaatgggcagccggagaacaactacaagaccacgcctcccgtgctggactccgacggctccttcttcctctacagcaggctaaccgtggacaagagcaggtggcaggaggggaatgtcttctcatgctccgtgatgcatgaggctctgcacaaccactacacacagaagagcctctccctgtctctgggtaaa

SEQ ID NO: 18 - protein, 377 aa, Artificial Sequence
  Description of Artificial Sequence: Synthetic polypeptide
  IL-22 Fc fusion IgG4 (full) N297A
APISSHCRLDKSNFQQPYITNRTFMLAKEASLADNNTDVRLIGEKLFHGVSMSERCYLMKQVLNFTLEEVLFPQSDRFQPYMQEVVPFLARLSNRLSTCHIEGDDLHIQRNVQKLKDTVKKLGESGEIKAIGELDLLFMSLRNACIRVESKYGPPCPPCPAPEFLGGPSVFLFPPKPKDTLMISRTPEVTCVVVDVSQEDPEVQFNWYVDGVEVHNAKTKPREEQFASTYRVVSVLTVLHQDWLNGKEYKCKVSNKGLPSSIEKTISKAKGQPREPQVYTLPPSQEEMTKNQVSLTCLVKGFYPSDIAVEWESNGQPENNYKTTPPVLDSDGSFFLYSRLTVDKSRWQEGNVFSCSVMHEALHNHYTQKSLSLSLGK

SEQ ID NO: 19 - DNA, 1134 bp, Artificial Sequence
  Description of Artificial Sequence: Synthetic polynucleotide
  IL-22 Fc fusion IgG1 (full) N297G
gcgcccatcagctcccactgcaggcttgacaagtccaacttccagcagccctatatcaccaaccgcaccttcatgctggctaaggaggctagcttggctgataacaacacagacgttcgtctcattggggagaaactgttccacggagtcagtatgagtgagcgctgctatctgatgaagcaggtgctgaacttcacccttgaagaagtgctgttccctcaatctgataggttccagccttatatgcaggaggtggtgcccttcctggccaggctcagcaacaggctaagcacatgtcatattgaaggtgatgacctgcatatccagaggaatgtgcaaaagctgaaggacacagtgaaaaagcttggagagagtggagagatcaaagcaattggagaactggatttgctgtttatgtctctgagaaatgcctgcattgagcccaaatctagtgacaaaactcacacatgcccaccgtgcccagcacctgaactcctggggggaccgtcagtcttcctcttccccccaaaacccaaggacaccctcatgatctcccggacccctgaggtcacatgcgtggtggtggacgtgagccacgaagaccctgaggtcaagttcaactggtacgtggacggcgtggaggtgcataatgccaagacaaagccgcgggaggagcagtacggaagcacgtaccgtgtggtcagcgtcctcaccgtcctgcaccaggactggctgaatggcaaggagtacaagtgcaaggtctccaacaaagccctcccagcccccatcgagaaaaccatctccaaagccaaagggcagccccgagaaccacaggtgtacaccctgcccccatcccgggaagagatgaccaagaaccaggtcagcctgacctgcctggtcaaaggcttctatcccagcgacatcgccgtggagtgggagagcaatgggcagccggagaacaactacaagaccacgcctcccgtgctggactccgacggctccttcttcctctacagcaagctcaccgtggacaagagcaggtggcagcaggggaacgtcttctcatgctccgtgatgcatgaggctctgcacaaccactacacgcagaagagcctctccctgtctccgggtaaa

SEQ ID NO: 20 - protein, 378 aa, Artificial Sequence
  Description of Artificial Sequence: Synthetic polypeptide
  IL-22 Fc fusion IgG1 (full) N297G
APISSHCRLDKSNFQQPYITNRTFMLAKEASLADNNTDVRLIGEKLFHGVSMSERCYLMKQVLNFTLEEVLFPQSDRFQPYMQEVVPFLARLSNRLSTCHIEGDDLHIQRNVQKLKDTVKKLGESGEIKAIGELDLLFMSLRNACIEPKSSDKTHTCPPCPAPELLGGPSVFLFPPKPKDTLMISRTPEVTCVVVDVSHEDPEVKFNWYVDGVEVHNAKTKPREEQYGSTYRVVSVLTVLHQDWLNGKEYKCKVSNKALPAPIEKTISKAKGQPREPQVYTLPPSREEMTKNQVSLTCLVKGFYPSDIAVEWESNGQPENNYKTTPPVLDSDGSFFLYSKLTVDKSRWQQGNVFSCSVMHEALHNHYTQKSLSLSPGK

SEQ ID NO: 21 - DNA, 1134 bp, Artificial Sequence
  Description of Artificial Sequence: Synthetic polynucleotide
  IL-22 Fc fusion IgG1 (full) N297A
gcgcccatcagctcccactgcaggcttgacaagtccaacttccagcagccctatatcaccaaccgcaccttcatgctggctaaggaggctagcttggctgataacaacacagacgttcgtctcattggggagaaactgttccacggagtcagtatgagtgagcgctgctatctgatgaagcaggtgctgaacttcacccttgaagaagtgctgttccctcaatctgataggttccagccttatatgcaggaggtggtgcccttcctggccaggctcagcaacaggctaagcacatgtcatattgaaggtgatgacctgcatatccagaggaatgtgcaaaagctgaaggacacagtgaaaaagcttggagagagtggagagatcaaagcaattggagaactggatttgctgtttatgtctctgagaaatgcctgcattgagcccaaatctagtgacaaaactcacacatgcccaccgtgcccagcacctgaactcctggggggaccgtcagtcttcctcttccccccaaaacccaaggacaccctcatgatctcccggacccctgaggtcacatgcgtggtggtggacgtgagccacgaagaccctgaggtcaagttcaactggtacgtggacggcgtggaggtgcataatgccaagacaaagccgcgggaggagcagtacgctagcacgtaccgtgtggtcagcgtcctcaccgtcctgcaccaggactggctgaatggcaaggagtacaagtgcaaggtctccaacaaagccctcccagcccccatcgagaaaaccatctccaaagccaaagggcagccccgagaaccacaggtgtacaccctgcccccatcccgggaagagatgaccaagaaccaggtcagcctgacctgcctggtcaaaggcttctatcccagcgacatcgccgtggagtgggagagcaatgggcagccggagaacaactacaagaccacgcctcccgtgctggactccgacggctccttcttcctctacagcaagctcaccgtggacaagagcaggtggcagcaggggaacgtcttctcatgctccgtgatgcatgaggctctgcacaaccactacacgcagaagagcctctccctgtctccgggtaaa

SEQ ID NO: 22 - protein, 378 aa, Artificial Sequence
  Description of Artificial Sequence: Synthetic polypeptide
  IL-22 Fc fusion IgG1 (full) N297A
APISSHCRLDKSNFQQPYITNRTFMLAKEASLADNNTDVRLIGEKLFHGVSMSERCYLMKQVLNFTLEEVLFPQSDRFQPYMQEVVPFLARLSNRLSTCHIEGDDLHIQRNVQKLKDTVKKLGESGEIKAIGELDLLFMSLRNACIEPKSSDKTHTCPPCPAPELLGGPSVFLFPPKPKDTLMISRTPEVTCVVVDVSHEDPEVKFNWYVDGVEVHNAKTKPREEQYASTYRVVSVLTVLHQDWLNGKEYKCKVSNKALPAPIEKTISKAKGQPREPQVYTLPPSREEMTKNQVSLTCLVKGFYPSDIAVEWESNGQPENNYKTTPPVLDSDGSFFLYSKLTVDKSRWQQGNVFSCSVMHEALHNHYTQKSLSLSPGK

SEQ ID NO: 23 - DNA, 1128 bp, Artificial Sequence
  Description of Artificial Sequence: Synthetic polynucleotide
  IL-22 Fc fusion IgG4 (wt N297, minus Lys)
gcgcccatcagctcccactgcaggcttgacaagtccaacttccagcagccctatatcaccaaccgcaccttcatgctggctaaggaggctagcttggctgataacaacacagacgttcgtctcattggggagaaactgttccacggagtcagtatgagtgagcgctgctatctgatgaagcaggtgctgaacttcacccttgaagaagtgctgttccctcaatctgataggttccagccttatatgcaggaggtggtgcccttcctggccaggctcagcaacaggctaagcacatgtcatattgaaggtgatgacctgcatatccagaggaatgtgcaaaagctgaaggacacagtgaaaaagcttggagagagtggagagatcaaagcaattggagaactggatttgctgtttatgtctctgagaaatgcctgcattcgcgttgagtccaaatatggtcccccatgcccaccatgcccagcacctgagttcctggggggaccatcagtcttcctgttccccccaaaacccaaggacactctcatgatctcccggacccctgaggtcacgtgcgtggtggtggacgtgagccaggaagaccccgaggtccagttcaactggtacgtggatggcgtggaggtgcataatgccaagacaaagccgcgggaggagcagttcaacagcacgtaccgtgtggtcagcgtcctcaccgtcctgcaccaggactggctgaacggcaaggagtacaagtgcaaggtctccaacaaaggcctcccgtcctccatcgagaaaaccatctccaaagccaaagggcagccccgagagccacaggtgtacaccctgcccccatcccaggaggagatgaccaagaaccaggtcagcctgacctgcctggtcaaaggcttctaccccagcgacatcgccgtggagtgggagagcaatgggcagccggagaacaactacaagaccacgcctcccgtgctggactccgacggctccttcttcctctacagcaggctaaccgtggacaagagcaggtggcaggaggggaatgtcttctcatgctccgtgatgcatgaggctctgcacaaccactacacacagaagagcctctccctgtctctgggt

SEQ ID NO: 24 - protein, 376 aa, Artificial Sequence
  Description of Artificial Sequence: Synthetic polypeptide
  IL-22 Fc fusion IgG4 (wt N297, minus Lys)
APISSHCRLDKSNFQQPYITNRTFMLAKEASLADNNTDVRLIGEKLFHGVSMSERCYLMKQVLNFTLEEVLFPQSDRFQPYMQEVVPFLARLSNRLSTCHIEGDDLHIQRNVQKLKDTVKKLGESGEIKAIGELDLLFMSLRNACIRVESKYGPPCPPCPAPEFLGGPSVFLFPPKPKDTLMISRTPEVTCVVVDVSQEDPEVQFNWYVDGVEVHNAKTKPREEQFNSTYRVVSVLTVLHQDWLNGKEYKCKVSNKGLPSSIEKTISKAKGQPREPQVYTLPPSQEEMTKNQVSLTCLVKGFYPSDIAVEWESNGQPENNYKTTPPVLDSDGSFFLYSRLTVDKSRWQEGNVFSCSVMHEALHNHYTQKSLSLSLG

SEQ ID NO: 25 - DNA, 1131 bp, Artificial Sequence
  Description of Artificial Sequence: Synthetic polynucleotide
  IL-22 Fc fusion IgG1 (wt N297, minus Lys)
gcgcccatcagctcccactgcaggcttgacaagtccaacttccagcagccctatatcaccaaccgcaccttcatgctggctaaggaggctagcttggctgataacaacacagacgttcgtctcattggggagaaactgttccacggagtcagtatgagtgagcgctgctatctgatgaagcaggtgctgaacttcacccttgaagaagtgctgttccctcaatctgataggttccagccttatatgcaggaggtggtgcccttcctggccaggctcagcaacaggctaagcacatgtcatattgaaggtgatgacctgcatatccagaggaatgtgcaaaagctgaaggacacagtgaaaaagcttggagagagtggagagatcaaagcaattggagaactggatttgctgtttatgtctctgagaaatgcctgcattgagcccaaatctagtgacaaaactcacacatgcccaccgtgcccagcacctgaactcctggggggaccgtcagtcttcctcttccccccaaaacccaaggacaccctcatgatctcccggacccctgaggtcacatgcgtggtggtggacgtgagccacgaagaccctgaggtcaagttcaactggtacgtggacggcgtggaggtgcataatgccaagacaaagccgcgggaggagcagtacaacagcacgtaccgtgtggtcagcgtcctcaccgtcctgcaccaggactggctgaatggcaaggagtacaagtgcaaggtctccaacaaagccctcccagcccccatcgagaaaaccatctccaaagccaaagggcagccccgagaaccacaggtgtacaccctgcccccatcccgggaagagatgaccaagaaccaggtcagcctgacctgcctggtcaaaggcttctatcccagcgacatcgccgtggagtgggagagcaatgggcagccggagaacaactacaagaccacgcctcccgtgctggactccgacggctccttcttcctctacagcaagctcaccgtggacaagagcaggtggcagcaggggaacgtcttctcatgctccgtgatgcatgaggctctgcacaaccactacacgcagaagagcctctccctgtctccgggt

SEQ ID NO: 26 - protein, 377 aa, Artificial Sequence
  Description of Artificial Sequence: Synthetic polypeptide
  IL-22 Fc fusion IgG1 (wt N297, minus Lys)
APISSHCRLDKSNFQQPYITNRTFMLAKEASLADNNTDVRLIGEKLFHGVSMSERCYLMKQVLNFTLEEVLFPQSDRFQPYMQEVVPFLARLSNRLSTCHIEGDDLHIQRNVQKLKDTVKKLGESGEIKAIGELDLLFMSLRNACIEPKSSDKTHTCPPCPAPELLGGPSVFLFPPKPKDTLMISRTPEVTCVVVDVSHEDPEVKFNWYVDGVEVHNAKTKPREEQYNSTYRVVSVLTVLHQDWLNGKEYKCKVSNKALPAPIEKTISKAKGQPREPQVYTLPPSREEMTKNQVSLTCLVKGFYPSDIAVEWESNGQPENNYKTTPPVLDSDGSFFLYSKLTVDKSRWQQGNVFSCSVMHEALHNHYTQKSLSLSPG

SEQ ID NO: 27 - DNA, 1131 bp, Artificial Sequence
  Description of Artificial Sequence: Synthetic polynucleotide
  IL-22 Fc fusion IgG4 (N297 wt)
gcgcccatcagctcccactgcaggcttgacaagtccaacttccagcagccctatatcaccaaccgcaccttcatgctggctaaggaggctagcttggctgataacaacacagacgttcgtctcattggggagaaactgttccacggagtcagtatgagtgagcgctgctatctgatgaagcaggtgctgaacttcacccttgaagaagtgctgttccctcaatctgataggttccagccttatatgcaggaggtggtgcccttcctggccaggctcagcaacaggctaagcacatgtcatattgaaggtgatgacctgcatatccagaggaatgtgcaaaagctgaaggacacagtgaaaaagcttggagagagtggagagatcaaagcaattggagaactggatttgctgtttatgtctctgagaaatgcctgcattcgcgttgagtccaaatatggtcccccatgcccaccatgcccagcacctgagttcctggggggaccatcagtcttcctgttccccccaaaacccaaggacactctcatgatctcccggacccctgaggtcacgtgcgtggtggtggacgtgagccaggaagaccccgaggtccagttcaactggtacgtggatggcgtggaggtgcataatgccaagacaaagccgcgggaggagcagttcaacagcacgtaccgtgtggtcagcgtcctcaccgtcctgcaccaggactggctgaacggcaaggagtacaagtgcaaggtctccaacaaaggcctcccgtcctccatcgagaaaaccatctccaaagccaaagggcagccccgagagccacaggtgtacaccctgcccccatcccaggaggagatgaccaagaaccaggtcagcctgacctgcctggtcaaaggcttctaccccagcgacatcgccgtggagtgggagagcaatgggcagccggagaacaactacaagaccacgcctcccgtgctggactccgacggctccttcttcctctacagcaggctaaccgtggacaagagcaggtggcaggaggggaatgtcttctcatgctccgtgatgcatgaggctctgcacaaccactacacacagaagagcctctccctgtctctgggtaaa

SEQ ID NO: 28 - protein, 377 aa, Artificial Sequence
  Description of Artificial Sequence: Synthetic polypeptide
  IL-22 Fc fusion IgG4 (N297 wt)
APISSHCRLDKSNFQQPYITNRTFMLAKEASLADNNTDVRLIGEKLFHGVSMSERCYLMKQVLNFTLEEVLFPQSDRFQPYMQEVVPFLARLSNRLSTCHIEGDDLHIQRNVQKLKDTVKKLGESGEIKAIGELDLLFMSLRNACIRVESKYGPPCPPCPAPEFLGGPSVFLFPPKPKDTLMISRTPEVTCVVVDVSQEDPEVQFNWYVDGVEVHNAKTKPREEQFNSTYRVVSVLTVLHQDWLNGKEYKCKVSNKGLPSSIEKTISKAKGQPREPQVYTLPPSQEEMTKNQVSLTCLVKGFYPSDIAVEWESNGQPENNYKTTPPVLDSDGSFFLYSRLTVDKSRWQEGNVFSCSVMHEALHNHYTQKSLSLSLGK

SEQ ID NO: 29 - DNA, 1134 bp, Artificial Sequence
  Description of Artificial Sequence: Synthetic polynucleotide
  IL-22 Fc fusion IgG1 (N297 wt)
gcgcccatcagctcccactgcaggcttgacaagtccaacttccagcagccctatatcaccaaccgcaccttcatgctggctaaggaggctagcttggctgataacaacacagacgttcgtctcattggggagaaactgttccacggagtcagtatgagtgagcgctgctatctgatgaagcaggtgctgaacttcacccttgaagaagtgctgttccctcaatctgataggttccagccttatatgcaggaggtggtgcccttcctggccaggctcagcaacaggctaagcacatgtcatattgaaggtgatgacctgcatatccagaggaatgtgcaaaagctgaaggacacagtgaaaaagcttggagagagtggagagatcaaagcaattggagaactggatttgctgtttatgtctctgagaaatgcctgcattgagcccaaatctagtgacaaaactcacacatgcccaccgtgcccagcacctgaactcctggggggaccgtcagtcttcctcttccccccaaaacccaaggacaccctcatgatctcccggacccctgaggtcacatgcgtggtggtggacgtgagccacgaagaccctgaggtcaagttcaactggtacgtggacggcgtggaggtgcataatgccaagacaaagccgcgggaggagcagtacaacagcacgtaccgtgtggtcagcgtcctcaccgtcctgcaccaggactggctgaatggcaaggagtacaagtgcaaggtctccaacaaagccctcccagcccccatcgagaaaaccatctccaaagccaaagggcagccccgagaaccacaggtgtacaccctgcccccatcccgggaagagatgaccaagaaccaggtcagcctgacctgcctggtcaaaggcttctatcccagcgacatcgccgtggagtgggagagcaatgggcagccggagaacaactacaagaccacgcctcccgtgctggactccgacggctccttcttcctctacagcaagctcaccgtggacaagagcaggtggcagcaggggaacgtcttctcatgctccgtgatgcatgaggctctgcacaaccactacacgcagaagagcctctccctgtctccgggtaaa

SEQ ID NO: 30 - protein, 378 aa, Artificial Sequence
  Description of Artificial Sequence: Synthetic polypeptide
  IL-22 Fc fusion IgG1 (N297 wt)
APISSHCRLDKSNFQQPYITNRTFMLAKEASLADNNTDVRLIGEKLFHGVSMSERCYLMKQVLNFTLEEVLFPQSDRFQPYMQEVVPFLARLSNRLSTCHIEGDDLHIQRNVQKLKDTVKKLGESGEIKAIGELDLLFMSLRNACIEPKSSDKTHTCPPCPAPELLGGPSVFLFPPKPKDTLMISRTPEVTCVVVDVSHEDPEVKFNWYVDGVEVHNAKTKPREEQYNSTYRVVSVLTVLHQDWLNGKEYKCKVSNKALPAPIEKTISKAKGQPREPQVYTLPPSREEMTKNQVSLTCLVKGFYPSDIAVEWESNGQPENNYKTTPPVLDSDGSFFLYSKLTVDKSRWQQGNVFSCSVMHEALHNHYTQKSLSLSPGK

SEQ ID NO: 31 - protein, 5 aa, Artificial Sequence
  Description of Artificial Sequence: Synthetic hinge peptide
CPPCP

SEQ ID NO: 32 - protein, 5 aa, Artificial Sequence
  Description of Artificial Sequence: Synthetic linker peptide
DKTHT

SEQ ID NO: 33 - protein, 10 aa, Artificial Sequence
  Description of Artificial Sequence: Synthetic linker peptide
EPKSCDKTHT

SEQ ID NO: 34 - protein, 11 aa, Artificial Sequence
  Description of Artificial Sequence: Synthetic linker peptide
VEPKSCDKTHT

SEQ ID NO: 35 - protein, 12 aa, Artificial Sequence
  Description of Artificial Sequence: Synthetic linker peptide
KVEPKSCDKTHT

SEQ ID NO: 36 - protein, 13 aa, Artificial Sequence
  Description of Artificial Sequence: Synthetic linker peptide
KKVEPKSCDKTHT

SEQ ID NO: 37 - protein, 14 aa, Artificial Sequence
  Description of Artificial Sequence: Synthetic linker peptide
DKKVEPKSCDKTHT

SEQ ID NO: 38 - protein, 15 aa, Artificial Sequence
  Description of Artificial Sequence: Synthetic linker peptide
VDKKVEPKSCDKTHT

SEQ ID NO: 39 - protein, 16 aa, Artificial Sequence
  Description of Artificial Sequence: Synthetic linker peptide
KVDKKVEPKSCDKTHT

SEQ ID NO: 40 - protein, 10 aa, Artificial Sequence
  Description of Artificial Sequence: Synthetic linker peptide
EPKSSDKTHT

SEQ ID NO: 41 - protein, 8 aa, Artificial Sequence
  Description of Artificial Sequence: Synthetic linker peptide
GGGDKTHT

SEQ ID NO: 42 - protein, 12 aa, Artificial Sequence
  Description of Artificial Sequence: Synthetic linker (IgG3) peptide
ELKTPLGDTTHT

SEQ ID NO: 43 - protein, 6 aa, Artificial Sequence
  Description of Artificial Sequence: Synthetic linker peptide
SKYGPP

SEQ ID NO: 44 - protein, 9 aa, Artificial Sequence
  Description of Artificial Sequence: Synthetic linker peptide
RVESKYGPP

SEQ ID NO: 45 - protein, 3 aa, Artificial Sequence
  Description of Artificial Sequence: Synthetic linker peptide
GGS

SEQ ID NO: 46 - protein, 4 aa, Artificial Sequence
  Description of Artificial Sequence: Synthetic linker peptide
GGGS

SEQ ID NO: 47 - protein, 5 aa, Artificial Sequence
  Description of Artificial Sequence: Synthetic linker peptide
GGGGS

SEQ ID NO: 48 - protein, 146 aa, Pan troglodytes
APISSHCRLDKSSFQQPYITNRTFMLAKEASLADNNTDVRLIGEKLFHGVSMSERCYLMKQVLNFTLEEVLFPQSDRFQPYMQEVVPFLARLSNRLSTCHIEGDDLHIQRNVQKLKDTVKKLGENGEIKAIGELDLLFMSLRNACI

SEQ ID NO: 49 - protein, 146 aa, Pongo abelii
APISSHCRLDKSNFQQPYITNRTFMLAKEASLADNNTDVRLIGEKLFRGVSMSERCYLMKQVLNFTLEEVLFPQSDRFQPYMQEVVPFLARLSNRLSTCHIEGDDLHIQRNVQKLKDTVKKLGESGEIKAIGELDLLFMSLRNACI

SEQ ID NO: 50 - protein, 146 aa, Mus musculus
LPVNTRCKLEVSNFQQPYIVNRTFMLAKEASLADNNTDVRLIGEKLFRGVSAKDQCYLMKQVLNFTLEDVLLPQSDRFQPYMQEVVPFLTKLSNQLSSCHISGDDQNIQKNVRRLKETVKKLGESGEIKAIGELDLLFMSLRNACV

SEQ ID NO: 51 - protein, 146 aa, Canis familiaris
LPISSHCRLDKSNFQQPYITNRTFMLAKEASLADNNTDVRLIGEKLFHGVNMGERCYLMKEVLNFTLEEVLLPQSDRFQPYMQEVVPFLARLSNKLSQCHIENDDQHIQRNVQKLKDTVQKLGENGEIKAIGELDLLFMALRNACV

SEQ ID NO: 52 - DNA, 94 bp, Artificial Sequence
  Description of Artificial Sequence: Synthetic IL-22 Fc fusion protein IgG1 forward primer
ttgaattccaccatgggatggtcatgtatcatcctttttctagtagcaactgcaactggagtacattcagcgcccatcagctcccactgcaggc

SEQ ID NO: 53 - DNA, 33 bp, Artificial Sequence
  Description of Artificial Sequence: Synthetic IL-22 Fc fusion IgG1 reverse primer
aggtcgactcatttacccggagacagggagagg

SEQ ID NO: 54 - DNA, 94 bp, Artificial Sequence; identical to SEQ ID NO: 52
  Description of Artificial Sequence: Synthetic IL-22 Fc fusion IgG4 forward primer

SEQ ID NO: 55 - DNA, 33 bp, Artificial Sequence
  Description of Artificial Sequence: Synthetic IL-22 Fc fusion IgG4 reverse primer
aggtcgacttatttacccagagacagggagagg

SEQ ID NO: 56 - DNA, 35 bp, Artificial Sequence
  Description of Artificial Sequence: Synthetic IgG1 N297G forward primer
gcgggaggagcagtacggaagcacgtaccgtgtgg

SEQ ID NO: 57 - DNA, 35 bp, Artificial Sequence
  Description of Artificial Sequence: Synthetic IgG1 N297G reverse primer
ccacacggtacgtgcttccgtactgctcctcccgc

SEQ ID NO: 58 - DNA, 51 bp, Artificial Sequence
  Description of Artificial Sequence: Synthetic IgG4 N297G forward primer
acaaagccgcgggaggagcagttcggaagcacgtaccgtgtggtcagcgtc

SEQ ID NO: 59 - DNA, 51 bp, Artificial Sequence
  Description of Artificial Sequence: Synthetic IgG4 N297G reverse primer
gacgctgaccacacggtacgtgcttccgaactgctcctcccgcggctttgt

SEQ ID NO: 60 - protein, 411 aa, Artificial Sequence
  Description of Artificial Sequence: Synthetic polypeptide
  IL-22 Fc fusion IgG2a
MAVLQKSMSFSLMGTLAASCLLLIALWAQEANALPVNTRCKLEVSNFQQPYIVNRTFMLAKEASLADNNTDVRLIGEKLFRGVSAKDQCYLMKQVLNFTLEDVLLPQSDRFQPYMQEVVPFLTKLSNQLSSCHISGDDQNIQKNVRRLKETVKKLGESGEIKAIGELDLLFMSLRNACVARGPTIKPCPPCKCPAPNLLGGPSVFIFPPKIKDVLMISLSPIVTCVVVDVSEDDPDVQISWFVNNVEVHTAQTQTHREDYNSTLRVVSALPIQHQDWMSGKEFKCKVNNKDLPAPIERTISKPKGSVRAPQVYVLPPPEEEMTKKQVTLTCMVTDFMPEDIYVEWTNNGKTELNYKNTEPVLDSDGSYFMYSKLRVEKKNWVERNSYSCSVVHEGLHNHHTTKSFSRTPGK

SEQ ID NO: 61 - protein, 372 aa, Artificial Sequence
  Description of Artificial Sequence: Synthetic polypeptide
  IL-22 IgG1 fusion knob (T366W) minus Lys
APISSHCRLDKSNFQQPYITNRTFMLAKEASLADNNTDVRLIGEKLFHGVSMSERCYLMKQVLNFTLEEVLFPQSDRFQPYMQEVVPFLARLSNRLSTCHIEGDDLHIQRNVQKLKDTVKKLGESGEIKAIGELDLLFMSLRNACIDKTHTCPPCPAPELLGGPSVFLFPPKPKDTLMISRTPEVTCVVVDVSHEDPEVKFNWYVDGVEVHNAKTKPREEQYNSTYRVVSVLTVLHQDWLNGKEYKCKVSNKALPAPIEKTISKAKGQPREPQVYTLPPSREEMTKNQVSLWCLVKGFYPSDIAVEWESNGQPENNYKTTPPVLDSDGSFFLYSKLTVDKSRWQQGNVFSCSVMHEALHNHYTQKSLSLSPG

SEQ ID NO: 62 - protein, 226 aa, Artificial Sequence
  Description of Artificial Sequence: Synthetic polypeptide
  Monomeric Fc hole
DKTHTCPPCPAPELLGGPSVFLFPPKPKDTLMISRTPEVTCVVVDVSHEDPEVKFNWYVDGVEVHNAKTKPREEQYNSTYRVVSVLTVLHQDWLNGKEYKCKVSNKALPAPIEKTISKAKGQPREPQVYTLPPSREEMTKNQVSLSCAVKGFYPSDIAVEWESNGQPENNYKTTPPVLDSDGSFFLVSKLTVDKSRWQQGNVFSCSVMHEALHNHYTQKSLSLSPG

SEQ ID NO: 63 - protein, 7 aa, Artificial Sequence
  Description of Artificial Sequence: Synthetic linker peptide
GGGSTHT

SEQ ID NO: 64 - protein, 14 aa, Artificial Sequence
  Description of Artificial Sequence: Synthetic linker peptide
DKKVEPKSSDKTHT

SEQ ID NO: 65 - protein, 16 aa, Artificial Sequence
  Description of Artificial Sequence: Synthetic linker peptide
KVDKKVEPKSSDKTHT

SEQ ID NO: 66 - protein, 13 aa, Artificial Sequence
  Description of Artificial Sequence: Synthetic linker peptide
KKVEPKSSDKTHT

SEQ ID NO: 67 - protein, 11 aa, Artificial Sequence
  Description of Artificial Sequence: Synthetic linker peptide
VEPKSSDKTHT

SEQ ID NO: 68 - protein, 12 aa, Artificial Sequence
  Description of Artificial Sequence: Synthetic linker peptide
KVEPKSSDKTHT

SEQ ID NO: 69 - protein, 15 aa, Artificial Sequence
  Description of Artificial Sequence: Synthetic linker peptide
VDKKVEPKSSDKTHT

SEQ ID NO: 70 - DNA, 1152 bp, Homo sapiens
  CDS (58)..(597)
cttcagaacaggttctccttccccagtcaccagttgctcgagttagaattgtctgcaatggccgccctgcagaaatctgtgagctctttccttatggggaccctggccaccagctgcctccttctcttggccctcttggtacagggaggagcagctgcgcccatcagctcccactgcaggcttgacaagtccaacttccagcagccctatatcaccaaccgcaccttcatgctggctaaggaggctagcttggctgataacaacacagacgttcgtctcattggggagaaactgttccacggagtcagtatgagtgagcgctgctatctgatgaagcaggtgctgaacttcacccttgaagaagtgctgttccctcaatctgataggttccagccttatatgcaggaggtggtgcccttcctggccaggctcagcaacaggctaagcacatgtcatattgaaggtgatgacctgcatatccagaggaatgtgcaaaagctgaaggacacagtgaaaaagcttggagagagtggagagatcaaagcaattggagaactggatttgctgtttatgtctctgagaaatgcctgcatttgaccagagcaaagctgaaaaatgaataactaaccccctttccctgctagaaataacaattagatgccccaaagcgattttttttaaccaaaaggaagatgggaagccaaactccatcatgatgggtggattccaaatgaacccctgcgttagttacaaaggaaaccaatgccacttttgtttataagaccagaaggtagactttctaagcatagatatttattgataacatttcattgtaactggtgttctatacacagaaaacaatttattttttaaataattgtctttttccataaaaaagattactttccattcctttaggggaaaaaacccctaaatagcttcatgtttccataatcagtactttatatttataaatgtatttattattattataagactgcattttatttatatcattttattaatatggatttatttatagaaacatcattcgatattgctacttgagtgtaaggctaatattgatatttatgacaataattatagagctataacatgtttatttgacctcaataaacacttggatatccc

SEQ ID NO: 71 - protein, 179 aa, Homo sapiens
MAALQKSVSSFLMGTLATSCLLLLALLVQGGAAAPISSHCRLDKSNFQQPYITNRTFMLAKEASLADNNTDVRLIGEKLFHGVSMSERCYLMKQVLNFTLEEVLFPQSDRFQPYMQEVVPFLARLSNRLSTCHIEGDDLHIQRNVQKLKDTVKKLGESGEIKAIGELDLLFMSLRNACI

SEQ ID NO: 72 - DNA, 1236 bp, Artificial Sequence
  Synthetic polypeptide
atggctgtcctgcagaaatctatgagtttttcccttatggggactttggccgccagctgcctgcttctcattgccctgtgggcccaggaggcaaatgcgctgcccgtcaacacccggtgcaagcttgaggtgtccaacttccagcagccatacatcgtcaaccgcacctttatgctggccaaggaggccagccttgcagataacaacacagatgtccggctcatcggggagaaactgttccgaggagtcagtgctaaggatcagtgctacctgatgaagcaggtgctcaacttcaccctggaagacgttctgctcccccagtcagacaggttccagccctacatgcaggaggtggtgcctttcctgaccaaactcagcaatcagctcagctcctgtcacatcagcggtgacgaccagaacatccagaagaatgtcagaaggctgaaggagacagtgaaaaagcttggagagagtggagagatcaaggcgattggggaactggacctgctgtttatgtctctgagaaatgcttgcgtcgctcgaggacccacaatcaagccctgtcctccatgcaaatgcccagcacctaacctcttgggtggaccatccgtcttcatcttccctccaaagatcaaggatgtactcatgatctccctgagccccatagtcacatgtgtggtggtggatgtgagcgaggatgacccagatgtccagatcagctggtttgtgaacaacgtggaagtacacacagctcagacacaaacccatagagaggattacaacagtactctacgcgtggtcagtgccctccccatccagcaccaggactggatgagtggcaaggagttcaaatgcaaggtcaacaacaaagacctcccagcgcccatcgagagaaccatctcaaaacccaaagggtcagtaagagctccacaggtatatgtcttgcctccaccagaagaagagatgactaagaaacaggtcactctgacctgcatggtcacagacttcatgcctgaagacatttacgtggagtggaccaacaacgggaaaacagagctaaactacaagaacactgaaccagtcctggactctgatggttcttacttcatgtacagcaagctgagagtggaaaagaagaactgggtggaaagaaatagctactcctgttcagtggtccacgagggtctgcacaatcaccacacgactaagagcttctcccggactccgggtaaatga

SEQ ID NO: 73 - protein, 411 aa, Artificial Sequence; identical to SEQ ID NO: 60
  Synthetic polypeptide

SEQ ID NO: 74 - DNA, 20 bp, Artificial Sequence
  Synthetic primer
aggtccattcagatgctggt

SEQ ID NO: 75 - DNA, 20 bp, Artificial Sequence
  Synthetic primer
taggtgtggttgacgtggag

SEQ ID NO: 76 - DNA, 20 bp, Artificial Sequence
  Synthetic primer
ccaccccacactcacaccgg

SEQ ID NO: 77 - protein, 177 aa, Homo sapiens [sequence omitted]

SEQ ID NO: 78 - protein, 176 aa, Homo sapiens
MKASSLAFSLLSAAFYLLWTPSTGLKTLNLGSCVIATNLQEIRNGFSEIRGSVQAKDGNIDIRILRRTESLQDTKPANRCCLLRHLLRLYLDRVFKNYQTPDHYTLRKISSLANSFLTIKKDLRLCHAHMTCHCGEEAMKKYSQILSHFEKLEPQAAVVKALGELDILLQWMEETE

SEQ ID NO: 79 - protein, 207 aa, Homo sapiens
MNFQQRLQSLWTLASRPFCPPLLATASQMQMVVLPCLGFTLLLWSQVSGAQGQEFHFGPCQVKGVVPQKLWEAFWAVKDTMQAQDNITSARLLQQEVLQNVSDAESCYLVHTLLEFYLKTVFKNYHNRTVEVRTLKSFSTLANNFVLIVSQLQPSQENEMFSIRDSAHRRFLLFRRAFKQLDVEAALTKALGEVDILLTWMQKFYKL

SEQ ID NO: 80 - protein, 171 aa, Homo sapiens
MLVNFILRCGLLLVTLSLAIAKHKQSSFTKSCYPRGTLSQAVDALYIKAAWLKATIPEDRIKNIRLLKKKTKKQFMKNCQFQEQLLSFFMEDVFGQLQLQGCKKIRFVEDFHSLRQKLSHCISCASSAREMKSITRMKRIFYRIGNKGIYKAISELDILLSWIKKLLESSQ